European Patent Application EP 4 431 523 A1, published September 18, 2024. Title: PREPARATION FOR CHIMERIC ANTIGEN RECEPTOR IMMUNE CELL CONSTRUCTED ON BASIS OF GAS6 AND USE OF CHIMERIC ANTIGEN RECEPTOR IMMUNE CELL. Applicant: WEST CHINA HOSPITAL, SICHUAN UNIVERSITY. The sequence listing filed with the application follows.

SEQUENCE LISTING (9 sequences)

SEQ ID NO: 1 - protein, 678 aa, Homo sapiens
MAPSLSPGPAALRRAPQLLLLLLAAECALAALLPAREATQFLRPRQRRAFQVFEEAKQGHLERECVEELCSREEAREVFENDPETDYFYPRYLDCINKYGSPYTKNSGFATCVQNLPDQCTPNPCDRKGTQACQDLMGNFFCLCKAGWGGRLCDKDVNECSQENGGCLQICHNKPGSFHCSCHSGFELSSDGRTCQDIDECADSEACGEARCKNLPGSYSCLCDEGFAYSSQEKACRDVDECLQGRCEQVCVNSPGSYTCHCDGRGGLKLSQDMDTCEDILPCVPFSVAKSVKSLYLGRMFSGTPVIRLRFKRLQPTRLVAEFDFRTFDPEGILLFAGGHQDSTWIVLALRAGRLELQLRYNGVGRVTSSGPVINHGMWQTISVEELARNLVIKVNRDAVMKIAVAGDLFQPERGLYHLNLTVGGIPFHEKDLVQPINPRLDGCMRSWNWLNGEDTTIQETVKVNTRMQCFSVTERGSFYPGSGFAFYSLDYMRTPLDVGTESTWEVEVVAHIRPAADTGVLFALWAPDLRAVPLSVALVDYHSTKKLKKQLVVLAVEHTALALMEIKVCDGQEHVVTVSLRDGEATLEVDGTRGQSEVSAAQLQERLAVLERHLRSPVLTFAGGLPDVPVTSAPVTAFYRGCMTLEVNRRLLDLDEAAYKHSDITAHSCPPVEPAAA

SEQ ID NO: 2 - protein, 233 aa, synthetic construct
  source 1..233: note = mKate2
MSELIKENMHMKLYMEGTVNNHHFKCTSEGEGKPYEGTQTMRIKAVEGGPLPFAFDILATSFMYGSKTFINHTQGIPDFFKQSFPEGFTWERVTTYEDGGVLTATQDTSLQDGCLIYNVKIRGVNFPSNGPVMQKKTLGWEASTETLYPADGGLEGRADMALKLVGGGHLICNLKTTYRSKKPAKNLKMPGVYYVDRRLERIKEADKETYVEQHEVAVARYCDLPSKLGHKLN

SEQ ID NO: 3 - protein, 21 aa, synthetic construct
  source 1..21: note = signal peptite
MALPVTALLLPLALLLHAARP

SEQ ID NO: 4 - protein, 45 aa, synthetic construct
  source 1..45: note = CD8 hinge
TTTPAPRPPTPAPTIASQPLSLRPEACRPAAGGAVHTRGLDFACD

SEQ ID NO: 5 - protein, 24 aa, synthetic construct
  source 1..24: note = CD8 transmembrane domain
IYIWAPLAGTCGVLLLSLVITLYC

SEQ ID NO: 6 - protein, 43 aa, synthetic construct
  source 1..43: note = 4-1BB co-stimulatory region
KRGRKKLLYIFKQPFMRPVQTTQEEDGCSCRFPEEEEGGCELR

SEQ ID NO: 7 - protein, 111 aa, synthetic construct
  source 1..111: note = CD3 zeta cytoplasmic signal transduction sequence
VKFSRSADAPAYKQGQNQLYNELNLGRREEYDVLDKRRGRDPEMGGKPRRKNPQEGLYNELQKDKMAEAYSEIGMKGERRRGKGHDGLYQGLSTATKDTYDALHMQALPPR

SEQ ID NO: 8 - protein, 662 aa, synthetic construct
  source 1..662: note = CAR
MALPVTALLLPLALLLHAARPHCDGRGGLKLSQDMDTCEDILPCVPFSVAKSVKSLYLGRMFSGTPVIRLRFKRLQPTRLVAEFDFRTFDPEGILLFAGGHQDSTWIVLALRAGRLELQLRYNGVGRVTSSGPVINHGMWQTISVEELARNLVIKVNRDAVMKIAVAGDLFQPERGLYHLNLTVGGIPFHEKDLVQPINPRLDGCMRSWNWLNGEDTTIQETVKVNTRMQCFSVTERGSFYPGSGFAFYSLDYMRTPLDVGTESTWEVEVVAHIRPAADTGVLFALWAPDLRAVPLSVALVDYHSTKKLKKQLVVLAVEHTALALMEIKVCDGQEHVVTVSLRDGEATLEVDGTRGQSEVSAAQLQERLAVLERHLRSPVLTFAGGLPDVPVTSAPVTAFYRGCMTLEVNRRLLDLDEAAYKHSDITAHSCPPVEPAAATTTPAPRPPTPAPTIASQPLSLRPEACRPAAGGAVHTRGLDFACDIYIWAPLAGTCGVLLLSLVITLYCKRGRKKLLYIFKQPFMRPVQTTQEEDGCSCRFPEEEEGGCELRVKFSRSADAPAYKQGQNQLYNELNLGRREEYDVLDKRRGRDPEMGGKPRRKNPQEGLYNELQKDKMAEAYSEIGMKGERRRGKGHDGLYQGLSTATKDTYDALHMQALPPR

SEQ ID NO: 9 - DNA, 1986 bp, synthetic construct
  source 1..1986: mol_type = other DNA; note = CAR
atggccctgcccgtcaccgctctgctgctgccccttgctctgcttcttcatgcagcaaggccgcactgtgacgggcgtgggggcctcaagctgtcccaggacatggacacctgtgaggacatcttgccgtgcgtgcccttcagcgtggccaagagtgtgaagtccttgtacctgggccggatgttcagtgggacccccgtgatccgactgcgcttcaagaggctgcagcccaccaggctggtagctgagtttgacttccggacctttgaccccgagggcatcctcctctttgccggaggccaccaggacagcacctggatcgtgctggccctgagagccggccggctggagctgcagctgcgctacaacggtgtcggccgtgtcaccagcagcggcccggtcatcaaccatggcatgtggcagacaatctctgttgaggagctggcgcggaatctggtcatcaaggtcaacagggatgctgtcatgaaaatcgcggtggccggggacttgttccaaccggagcgaggactgtatcatctgaacctgaccgtgggaggtattcccttccatgagaaggacctcgtgcagcctataaaccctcgtctggatggctgcatgaggagctggaactggctgaacggagaagacaccaccatccaggaaacggtgaaagtgaacacgaggatgcagtgcttctcggtgacggagagaggctctttctaccccgggagcggcttcgccttctacagcctggactacatgcggacccctctggacgtcgggactgaatcaacctgggaagtagaagtcgtggctcacatccgcccagccgcagacacaggcgtgctgtttgcgctctgggcccccgacctccgtgccgtgcctctctctgtggcactggtagactatcactccacgaagaaactcaagaagcagctggtggtcctggccgtggagcatacggccttggccctaatggagatcaaggtctgcgacggccaagagcacgtggtcaccgtctcgctgagggacggtgaggccaccctggaggtggacggcaccaggggccagagcgaggtgagcgccgcgcagctgcaggagaggctggccgtgctcgagaggcacctgcggagccccgtgctcacctttgctggcggcctgccagatgtgccggtgacttcagcgccagtcaccgcgttctaccgcggctgcatgacactggaggtcaaccggaggctgctggacctggacgaggcggcgtacaagcacagcgacatcacggcccactcctgcccccccgtggagcccgccgcagccaccacgacgccagcgccgcgaccaccaacaccggcgcccaccatcgctagccagcccctgtccctgcgcccagaggcgtgccggccagcggcggggggcgcagtgcacacgagggggctggacttcgcctgtgatatctacatctgggcgcccttggccgggacttgtggggtccttctcctgtcactggttatcaccctttactgcaaacggggcagaaagaaactcctgtatatattcaaacaaccatttatgagaccagtacaaactactcaagaggaagatggctgtagctgccgatttccagaagaagaagaaggaggatgtgaactgagagtgaagttcagcaggagcgcagacgcccccgcgtacaagcagggccagaaccagctctataacgagctcaatctaggacgaagagaggagtacgatgttttggacaagagacgtggccgggaccctgagatggggggaaagccgagaaggaagaaccctcaggaaggcctgtacaatgaactgcagaaagataagatggcggaggcctacagtgagattgggatgaaaggcgagcgccggaggggcaaggggcacgatggcctttaccagggtctcagtacagccaccaaggacacctacgacgcccttcacatgcaggccctgccccctcgc